European Patent Application EP 4 691 565 A2, published February 11, 2026. Title: BISPECIFIC ANTIBODY AND USE THEREOF. Applicant: KEYMED BIOSCIENCES CO., LTD. Application EP. The sequence listing filed with the application follows.

SEQUENCE LISTING (105 sequences)

SEQ ID NO: 1 - protein, 306 aa, Homo sapiens
QSIKGNHLVKVYDYQEDGSVLLTCDAEAKNITWFKDGKMIGFLTEDKKKWNLGSNAKDPRGMYQCKGSQNKSKPLQVYYRMCQNCIELNAPEAAGGPSVFLFPPKPKDTLMISRTPEVTCVVVDVSHEDPEVKFNWYVDGVEVHNAKTKPREEQYNSTYRVVSVLTVLHQDWLNGKEYKCKVSNKALPASIEKTISKAKGQPREPQVCTLPPSRDELTKNQVSLSCAVKGFYPSDIAVEWESNGQPENNYKTTPPVLDSDGSFFLVSKLTVDKSRWQQGNVFSCSVMHEALHNHYTQKSLSLSPGK

SEQ ID NO: 2 - protein, 339 aa, Homo sapiens
QDGNEEMGGITQTPYKVSISGTTVILTCPQYPGSEILWQHNDKNIGGDEDDKNIGSDEDHLSLKEFSELEQSGYYVCYPRGSKPEDANFYLYLRARVCENCMEMDAPEAAGGPSVFLFPPKPKDTLMISRTPEVTCVVVDVSHEDPEVKFNWYVDGVEVHNAKTKPREEQYNSTYRVVSVLTVLHQDWLNGKEYKCKVSNKALPASIEKTISKAKGQPREPQVYTLPPCRDELTKNQVSLWCLVKGFYPSDIAVEWESNGQPENNYKTTPPVLDSDGSFFLYSKLTVDKSRWQQGNVFSCSVMHEALHNHYTQKSLSLSPGKGSGLNDIFEAQKIEWHE

SEQ ID NO: 3 - protein, 305 aa, Macaca fascicularis
QSFEENRKLNVYNQEDGSVLLTCHVKNTNITWFKEGKMIDILTAHKNKWNLGSNTKDPRGVYQCKGSKDKSKTLQVYYRMCQNCIELNAPEAAGGPSVFLFPPKPKDTLMISRTPEVTCVVVDVSHEDPEVKFNWYVDGVEVHNAKTKPREEQYNSTYRVVSVLTVLHQDWLNGKEYKCKVSNKALPASIEKTISKAKGQPREPQVCTLPPSRDELTKNQVSLSCAVKGFYPSDIAVEWESNGQPENNYKTTPPVLDSDGSFFLVSKLTVDKSRWQQGNVFSCSVMHEALHNHYTQKSLSLSPGK

SEQ ID NO: 4 - protein, 330 aa, Macaca fascicularis
QDGNEEMGSITQTPYQVSISGTTVILTCSQHLGSEAQWQHNGKNKEDSGDRLFLPEFSEMEQSGYYVCYPRGSNPEDASHHLYLKARVCENCMEMDAPEAAGGPSVFLFPPKPKDTLMISRTPEVTCVVVDVSHEDPEVKFNWYVDGVEVHNAKTKPREEQYNSTYRVVSVLTVLHQDWLNGKEYKCKVSNKALPASIEKTISKAKGQPREPQVYTLPPCRDELTKNQVSLWCLVKGFYPSDIAVEWESNGQPENNYKTTPPVLDSDGSFFLYSKLTVDKSRWQQGNVFSCSVMHEALHNHYTQKSLSLSPGKGSGLNDIFEAQKIEWHE

SEQ ID NO: 5 - protein, 109 aa, Homo sapiens
QAVVTQEPSLTVSPGGTVTLTCRSSTGAVTTSNYANWVQQKPGQAPRGLIGGTNKRAPWTPARFSGSLLGGKAALTLSGAQPEDEAEYYCALWYSNLWVFGGGTKLTVL

SEQ ID NO: 6 - DNA, 327 bp, Homo sapiens
  source 1..327: mol_type = other DNA
caggctgtggtcacacaagagcctagcctgacagtgtctcctggcggcacagtgaccctgacctgtagatcttctacaggcgccgtgaccaccagcaactacgctaattgggtgcagcagaagcccggccaggctcctagaggactgatcggcggaacaaacaagagagccccttggacacccgccagattctctggatctctgctcggcggaaaggccgctctgacactttctggtgctcagcctgaggacgaggccgagtactattgtgccctgtggtacagcaacctgtgggtgttcggcggaggcaccaaactgacagttctg

SEQ ID NO: 7 - protein, 14 aa, Homo sapiens
RSSTGAVTTSNYAN

SEQ ID NO: 8 - protein, 8 aa, Homo sapiens
GGTNKRAP

SEQ ID NO: 9 - protein, 9 aa, Homo sapiens
ALWYSNLWV

SEQ ID NO: 10 - protein, 109 aa, Homo sapiens
QAVVTQEPSLTVSPGGTVTLTCRSSTGAVTTSNYANWVQEKPGQAPRGLIGGTNKRAPWTPARFSGSLLGGKAALTLSGAQPEDEAEYYCALWYSNLWVFGGGTKLTVL

SEQ ID NO: 11 - DNA, 327 bp, Homo sapiens
  source 1..327: mol_type = other DNA
caggctgtggtcacacaagagcctagcctgacagtgtctcctggcggcacagtgaccctgacctgtagatcttctacaggcgccgtgaccaccagcaactacgctaattgggtgcaggagaagcccggccaggctcctagaggactgatcggcggaacaaacaagagagccccttggacacccgccagattctctggatctctgctcggcggaaaggccgctctgacactttctggtgctcagcctgaggacgaggccgagtactattgtgccctgtggtacagcaacctgtgggtgttcggcggaggcaccaaactgacagttctg

SEQ ID NO: 12 - protein, 109 aa, Homo sapiens
EAVVTQEPSLTVSPGGTVTLTCESSDGAVTTSNYANWVQEKPGQAPRGLIGGTNKEAPWTPARFSGSLLGGKAALTLSGAQPEDEAEYYCALWYSNLWVFGGGTKLTVL

SEQ ID NO: 13 - DNA, 327 bp, Homo sapiens
  source 1..327: mol_type = other DNA
gaggctgtggtcacacaagagcctagcctgacagtgtctcctggcggcacagtgaccctgacctgtgagtcttctgacggcgccgtgaccaccagcaactacgctaattgggtgcaggagaagcccggccaggctcctagaggactgatcggcggaacaaacaaggaggccccttggacacccgccagattctctggatctctgctcggcggaaaggccgctctgacactttctggtgctcagcctgaggacgaggccgagtactattgtgccctgtggtacagcaacctgtgggtgttcggcggaggcaccaaactgacagttctg

SEQ ID NO: 14 - protein, 14 aa, Homo sapiens
ESSDGAVTTSNYAN

SEQ ID NO: 15 - protein, 8 aa, Homo sapiens
GGTNKEAP

SEQ ID NO: 16 - protein, 109 aa, Homo sapiens
QAVVTQEPSLTVSPGGTVTLTCESSDGAVTTSNYANWVQEKPGQAPRGLIGGTNKEAPWTPARFSGSLLGGKAALTLSGAQPEDEAEYYCALWYSNLWVFGGGTKLTVL

SEQ ID NO: 17 - DNA, 327 bp, Homo sapiens
  source 1..327: mol_type = other DNA
caggctgtggtcacacaagagcctagcctgacagtgtctcctggcggcacagtgaccctgacctgtgagtcttctgacggcgccgtgaccaccagcaactacgctaattgggtgcaggagaagcccggccaggctcctagaggactgatcggcggaacaaacaaggaggccccttggacacccgccagattctctggatctctgctcggcggaaaggccgctctgacactttctggtgctcagcctgaggacgaggccgagtactattgtgccctgtggtacagcaacctgtgggtgttcggcggaggcaccaaactgacagttctg

SEQ ID NO: 18 - protein, 109 aa, Homo sapiens
QAVVTQEPSLTVSPGGTVTLTCRSSTGAVTTSNYANWVQEKPGQAPRGLIGGTNKRAPWTPARFSGSLLGGKAALTITGAQAEDEAEYYCVLWYSNLWVFGGGTKLTVL

SEQ ID NO: 19 - DNA, 327 bp, Homo sapiens
  source 1..327: mol_type = other DNA
caggctgtggtcacacaagagcctagcctgacagtgtctcctggcggcacagtgaccctgacctgtagatcttctacaggcgccgtgaccaccagcaactacgctaattgggtgcaggagaagcccggccaggctcctagaggactgatcggcggaacaaacaagagagccccttggacacccgccagattctctggatctctgctcggcggaaaggccgctctgacaatcactggtgctcaggctgaggacgaggccgagtactattgtgtgctgtggtacagcaacctgtgggtgttcggcggaggcaccaaactgacagttctg

SEQ ID NO: 20 - protein, 8 aa, Homo sapiens
YGTNKRAP

SEQ ID NO: 21 - protein, 9 aa, Homo sapiens
VLWYSNLWV

SEQ ID NO: 22 - protein, 109 aa, Homo sapiens
QAVVTQEPSLTVSPGGTVTLTCRSSTGAVTTSNYANWFQEKPGQAPRGLIYGTNKRAPWTPARFSGSLLGGKAALTLSGAQAEDEAEYYCVLWYSNLWVFGGGTKLTVL

SEQ ID NO: 23 - DNA, 327 bp, Homo sapiens
  source 1..327: mol_type = other DNA
caggctgtggtcacacaagagcctagcctgacagtgtctcctggcggcacagtgaccctgacctgtagatcttctacaggcgccgtgaccaccagcaactacgctaattggttccaggagaagcccggccaggctcctagaggactgatctacggaacaaacaagagagccccttggacacccgccagattctctggatctctgctcggcggaaaggccgctctgacactttctggtgctcaggctgaggacgaggccgagtactattgtgtcctgtggtacagcaacctgtgggtgttcggcggaggcaccaaactgacagttctg

SEQ ID NO: 24 - protein, 125 aa, Homo sapiens
EVQLVESGGGLVQPGGSLRLSCAASGFTFNTYAMNWVRQAPGKGLEWVSRIRSKYNNYATYYADSVKDRFTISRDDSKNTLYLQMNSLRAEDTAVYYCVRHGNFGNSYVSWFAYWGQGTLVTVSS

SEQ ID NO: 25 - DNA, 375 bp, Homo sapiens
  source 1..375: mol_type = other DNA
gaggtgcagctggttgaatctggcggaggactggttcagcctggcggatctctgagactgtcttgtgccgccagcggcttcaccttcaacacctacgctatgaactgggtccgacaggcccctggcaaaggactggaatgggtgtccagaatcaggtccaagtacaacaactacgccacctactacgccgacagcgtgaaggacagattcaccatcagcagggacgacagcaagaacaccctgtacctgcagatgaacagcctgagagccgaggacaccgccgtgtactactgtgtcagacacggcaacttcggcaacagctatgtgtcttggtttgcctactggggccagggcacactggtcacagttagctct

SEQ ID NO: 26 - protein, 6 aa, Homo sapiens
NTYAMN

SEQ ID NO: 27 - protein, 18 aa, Homo sapiens
IRSKYNNYATYYADSVKD

SEQ ID NO: 28 - protein, 14 aa, Homo sapiens
HGNFGNSYVSWFAY

SEQ ID NO: 29 - protein, 125 aa, Homo sapiens
EVQLVESGGGLVQPGGSLRLSCAASGFTFSTYAMNWVRKAPGKGLEWVSRIRSKYNNYATYYADSVKDRFTISRDDSKNTLYLQMNSLRAEDTAVYYCVRHGNFGNSYVSWFAYWGQGTLVTVSS

SEQ ID NO: 30 - DNA, 375 bp, Homo sapiens
  source 1..375: mol_type = other DNA
gaggtgcagctggttgaatctggcggaggactggttcagcctggcggatctctgagactgtcttgtgccgccagcggcttcaccttctccacctacgctatgaactgggtccgaaaggcccctggcaaaggactggaatgggtgtccagaatcaggtccaagtacaacaactacgccacctactacgccgacagcgtgaaggacagattcaccatcagcagggacgacagcaagaacaccctgtacctgcagatgaacagcctgagagccgaggacaccgccgtgtactactgtgtcagacacggcaacttcggcaacagctatgtgtcttggtttgcctactggggccagggcacactggtcacagttagctct

SEQ ID NO: 31 - protein, 6 aa, Homo sapiens
STYAMN

SEQ ID NO: 32 - protein, 125 aa, Homo sapiens
EVQLVESGGGLVQPGGSLRLSCAASGFTFSTYAMNWVRKAPGKGLEWVSRIRSKYNNYATYYADSVKDRFTISRDDSKNTLYLQMNSLRAEDTAVYYCVRHGNFGESYVSWFAYWGQGTLVTVSS

SEQ ID NO: 33 - DNA, 375 bp, Homo sapiens
  source 1..375: mol_type = other DNA
gaggtgcagctggttgaatctggcggaggactggttcagcctggcggatctctgagactgtcttgtgccgccagcggcttcaccttctccacctacgctatgaactgggtccgaaaggcccctggcaaaggactggaatgggtgtccagaatcaggtccaagtacaacaactacgccacctactacgccgacagcgtgaaggacagattcaccatcagcagggacgacagcaagaacaccctgtacctgcagatgaacagcctgagagccgaggacaccgccgtgtactactgtgtcagacacggcaacttcggcgagagctatgtgtcttggtttgcctactggggccagggcacactggtcacagttagctct

SEQ ID NO: 34 - protein, 14 aa, Homo sapiens
HGNFGESYVSWFAY

SEQ ID NO: 35 - protein, 125 aa, Homo sapiens
EVQLVESGGGLVQPGGSLRLSCAASGFTFSTYAMNWVRKAPGKGLEWVSRIRSKYNNYATYYADSVKDRFTISRDDSKNTLYLQMNSLRAEDTAVYYCVRHGNFGQSYVSWFAYWGQGTLVTVSS

SEQ ID NO: 36 - DNA, 375 bp, Homo sapiens
  source 1..375: mol_type = other DNA
gaggtgcagctggttgaatctggcggaggactggttcagcctggcggatctctgagactgtcttgtgccgccagcggcttcaccttctccacctacgctatgaactgggtccgaaaggcccctggcaaaggactggaatgggtgtccagaatcaggtccaagtacaacaactacgccacctactacgccgacagcgtgaaggacagattcaccatcagcagggacgacagcaagaacaccctgtacctgcagatgaacagcctgagagccgaggacaccgccgtgtactactgtgtcagacacggcaacttcggccagagctatgtgtcttggtttgcctactggggccagggcacactggtcacagttagctct

SEQ ID NO: 37 - protein, 14 aa, Homo sapiens
HGNFGQSYVSWFAY

SEQ ID NO: 38 - protein, 125 aa, Homo sapiens
EVQLVESGGGLVQPGGSLRLSCAASGFTFSTYAMNWVRKAPGKGLEWVSRIRSKYNNYATYYADSVKDRFTISRDDSKNTLYLQMNSLRAEDTAVYYCVRHGNFGDSYVSWFAYWGQGTLVTVSS

SEQ ID NO: 39 - DNA, 375 bp, Homo sapiens
  source 1..375: mol_type = other DNA
gaggtgcagctggttgaatctggcggaggactggttcagcctggcggatctctgagactgtcttgtgccgccagcggcttcaccttctccacctacgctatgaactgggtccgaaaggcccctggcaaaggactggaatgggtgtccagaatcaggtccaagtacaacaactacgccacctactacgccgacagcgtgaaggacagattcaccatcagcagggacgacagcaagaacaccctgtacctgcagatgaacagcctgagagccgaggacaccgccgtgtactactgtgtcagacacggcaacttcggcgacagctatgtgtcttggtttgcctactggggccagggcacactggtcacagttagctct

SEQ ID NO: 40 - protein, 14 aa, Homo sapiens
HGNFGDSYVSWFAY

SEQ ID NO: 41 - protein, 125 aa, Homo sapiens
EVQLVESGGGLVQPGGSLRLSCAASGFTFSTYAMNWVRKAPGKGLEWVSRIRSKYNNYATYYADSVKDRFTISRDDSKNTLYLQMNSLRAEDTAVYYCVRHGNFGTSYVSWFAYWGQGTLVTVSS

SEQ ID NO: 42 - DNA, 375 bp, Homo sapiens
  source 1..375: mol_type = other DNA
gaggtgcagctggttgaatctggcggaggactggttcagcctggcggatctctgagactgtcttgtgccgccagcggcttcaccttctccacctacgctatgaactgggtccgaaaggcccctggcaaaggactggaatgggtgtccagaatcaggtccaagtacaacaactacgccacctactacgccgacagcgtgaaggacagattcaccatcagcagggacgacagcaagaacaccctgtacctgcagatgaacagcctgagagccgaggacaccgccgtgtactactgtgtcagacacggcaacttcggcaccagctatgtgtcttggtttgcctactggggccagggcacactggtcacagttagctct

SEQ ID NO: 43 - protein, 14 aa, Homo sapiens
HGNFGTSYVSWFAY

SEQ ID NO: 44 - protein, 125 aa, Homo sapiens
EVQLVESGGGLVQPGGSLRLSCAASGFTFSDYAMNWVRKAPGKGLEWVSRIRSKYNNYATYYADSVEDRFTISRDDSKNTLYLQMNSLRAEDTAVYYCVRHGNFGNSYVSWFAYWGQGTLVTVSS

SEQ ID NO: 45 - DNA, 375 bp, Homo sapiens
  source 1..375: mol_type = other DNA
gaggtgcagctggttgaatctggcggaggactggttcagcctggcggatctctgagactgtcttgtgccgccagcggcttcaccttctccgactacgctatgaactgggtccgaaaggcccctggcaaaggactggaatgggtgtccagaatcaggtccaagtacaacaactacgccacctactacgccgacagcgtggaggacagattcaccatcagcagggacgacagcaagaacaccctgtacctgcagatgaacagcctgagagccgaggacaccgccgtgtactactgtgtcagacacggcaacttcggcaacagctatgtgtcttggtttgcctactggggccagggcacactggtcacagttagctct

SEQ ID NO: 46 - protein, 6 aa, Homo sapiens
SDYAMN

SEQ ID NO: 47 - protein, 18 aa, Homo sapiens
IRSKYNNYATYYADSVED

SEQ ID NO: 48 - protein, 125 aa, Homo sapiens
EVQLVESGGGLVQPGGSLRLSCAASGFTFNTYAMNWVRKAPGKGLEWVGRIRSKYNNYATYYADSVKDRFTISRDDSKNSLYLQMNSLKTEDTAVYYCARHGNFGNSYVSWFAYWGQGTLVTVSS

SEQ ID NO: 49 - DNA, 375 bp, Homo sapiens
  source 1..375: mol_type = other DNA
gaggtgcagctggttgaatctggcggaggactggttcagcctggcggatctctgagactgtcttgtgccgccagcggcttcaccttcaacacctacgctatgaactgggtccgaaaggcccctggcaaaggactggaatgggtgggaagaatcaggtccaagtacaacaactacgccacctactacgccgacagcgtgaaggacagattcaccatcagcagggacgacagcaagaacagcctgtacctgcagatgaacagcctgaaaaccgaggacaccgccgtgtactactgtgccagacacggcaacttcggcaacagctatgtgtcttggtttgcctactggggccagggcacactggtcacagttagctct

SEQ ID NO: 50 - protein, 125 aa, Homo sapiens
EVQLVESGGGLVQPGGSLRLSCAASGFTFNTYAMNWVRKAPGKGLEWVGRIRSKYNNYATYYADSVKDRFTISRDDSKNSLYLQMNSLKTEDTAVYYCVRHGNFGNSYVSWFAYWGQGTLVTVSS

SEQ ID NO: 51 - DNA, 375 bp, Homo sapiens
  source 1..375: mol_type = other DNA
gaggtgcagctggttgaatctggcggaggactggttcagcctggcggatctctgagactgtcttgtgccgccagcggcttcaccttcaacacctacgctatgaactgggtccgaaaggcccctggcaaaggactggaatgggtgggaagaatcaggtccaagtacaacaactacgccacctactacgccgacagcgtgaaggacagattcaccatcagcagggacgacagcaagaacagcctgtacctgcagatgaacagcctgaaaaccgaggacaccgccgtgtactactgtgtcagacacggcaacttcggcaacagctatgtgtcttggtttgcctactggggccagggcacactggtcacagttagctct

SEQ ID NO: 52 - protein, 125 aa, Homo sapiens
EVQLVESGGGLVQPGGSLRLSCAASGFTFNTYAMNWVRKAPGKGLEWVARIRSKYNNYATYYADSVKDRFTISRDDSKNSLYLQMNSLKTEDTAVYYCVRHGNFGNSYVSWFAYWGQGTLVTVSS

SEQ ID NO: 53 - DNA, 375 bp, Homo sapiens
  source 1..375: mol_type = other DNA
gaggtgcagctggttgaatctggcggaggactggttcagcctggcggatctctgagactgtcttgtgccgccagcggcttcaccttcaacacctacgctatgaactgggtccgaaaggcccctggcaaaggactggaatgggtggccagaatcaggtccaagtacaacaactacgccacctactacgccgacagcgtgaaggacagattcaccatcagcagggacgacagcaagaacagcctgtacctgcagatgaacagcctgaaaaccgaggacaccgccgtgtactactgtgtcagacacggcaacttcggcaacagctatgtgtcttggtttgcctactggggccagggcacactggtcacagttagctct

SEQ ID NO: 54 - protein, 214 aa, Homo sapiens
EIVLTQSPGTLSLSPGERATLSCRASQSVSSYLAWYQQKPGQAPRLLIYDASNRATGIPDRFSGSGSGTDFTLTISRLEPEDFAVYYCQQRSNWPITFGQGTKLEIKRTVAAPSVFIFPPSDEQLKSGTASVVCLLNNFYPREAKVQWKVDNALQSGNSQESVTEQDSKDSTYSLSSTLTLSKADYEKHKVYACEVTHQGLSSPVTKSFNRGEC

SEQ ID NO: 55 - DNA, 642 bp, Homo sapiens
  source 1..642: mol_type = other DNA
gagatcgtgctgacacagagccctggcacactgtcactgtctccaggcgagagagccacactgagctgtagagccagccagagcgtgtcctcttacctggcctggtatcagcagaagcctggacaggctcccagactgctgatctacgacgccagcaacagagccacaggcatccccgatagattcagcggctctggctctggcaccgacttcaccctgacaatcagcagactggaacccgaggacttcgccgtgtactactgccagcagagaagcaactggcccatcacattcggccagggcaccaagctggaaatcaagcgaactgtggctgcaccatctgtcttcatcttcccgccatctgatgagcagttgaaatctggaactgcctctgttgtgtgcctgctgaataacttctatcccagagaggccaaagtacagtggaaggtggataacgccctccaatcgggtaactcccaggagagtgtcacagagcaggacagcaaggacagcacctacagcctcagcagcaccctgacgctgagcaaagcagactacgagaaacacaaagtctacgcctgcgaagtcacccatcagggcctgagctcgcccgtcacaaagagcttcaacaggggagagtgt

SEQ ID NO: 56 - protein, 449 aa, Homo sapiens
EVQLLESGGGVVQPGGSLRLSCAASGFTFNDYAMHWVRQAPGKGLEWVSTISWNSGSIGYADSVKGRFTISRDNSKNTLYLQMNSLRAEDTAVYYCAKDIQYGNYYYGMDYWGQGTLVTVSSASTKGPSVFPLAPCSRSTSESTAALGCLVKDYFPEPVTVSWNSGALTSGVHTFPAVLQSSGLYSLSSVVTVPSSSLGTKTYTCNVDHKPSNTKVDKRVESKYGPPCPPCPAPEFEGGPSVFLFPPKPKDTLMISRTPEVTCVVVDVSQEDPEVQFNWYVDGVEVHNAKTKPREEQFNSTYRVVSVLTVLHQDWLNGKEYKCKVSNKGLASSIEKTISKAKGQPREPQVCTLPPSQEEMTKNQVSLSCAVKGFYPSDIAVEWESNGQPENNYKTTPPVLDSDGSFFLVSKLTVDKSRWQEGNVFSCSVMHEALHNHYTQKSLSLSLGK

SEQ ID NO: 57 - DNA, 1347 bp, Homo sapiens
  source 1..1347: mol_type = other DNA
gaagtgcagctgctggaatctggtggcggagttgttcagcctggcggctctctgagactgtcttgtgctgccagcggcttcaccttcaacgactacgctatgcactgggtccgacaggcccctggcaaaggacttgaatgggtgtccaccatcagctggaacagcggctctatcggctacgccgattccgtgaagggcagattcaccatctccagagacaacagcaagaacaccctgtacctgcagatgaacagcctgagagccgaggacaccgccgtgtactactgtgccaaggacatccagtacggcaactactactacggcatggactactggggccagggaacactggttaccgttagctctgctagcaccaagggccccagcgtgttccccctggccccttgcagcagaagcaccagcgagagcacagccgccctgggctgcctggtgaaggactacttccccgagcccgtgaccgtgtcctggaacagcggcgctctgaccagcggcgtgcataccttccccgccgtgctccagagcagcggactgtactccctgagcagcgtggtgaccgtgccttccagcagcctgggcaccaagacctacacctgcaacgtggaccacaagcccagcaacaccaaggtggacaagagagtggagagcaagtacggccctccctgccccccttgccctgcccccgagttcgagggcggacctagcgtgttcctgttcccccccaagcccaaggacaccctgatgatcagcagaacccccgaggtgacctgcgtggtggtggacgtgtcccaggaggaccccgaggtccagtttaattggtacgtggacggcgtggaagtgcataacgccaagaccaagcccagagaggagcagttcaacagcacctacagagtggtgtccgtgctgaccgtgctgcaccaggactggctgaacggcaaggaatacaagtgcaaggtctccaacaagggcctggccagcagcatcgagaagaccatcagcaaggccaagggccagccacgggagccccaggtctgcaccctgccacctagccaagaggagatgaccaagaaccaggtgtccctgagctgtgccgtgaaaggcttctatcccagcgatatcgccgtggagtgggagagcaacggccagcccgagaacaactacaagaccaccccccctgtgctggacagcgacggcagcttcttcctggtttccaagctgaccgtggacaagtccagatggcaggagggcaacgtcttcagctgctccgtgatgcacgaggccctgcacaaccactacacccagaagtccctgagcctgagcctgggcaag

SEQ ID NO: 58 - protein, 215 aa, Homo sapiens
QAVVTQEPSLTVSPGGTVTLTCRSSTGAVTTSNYANWVQQKPGQAPRGLIGGTNKRAPWTPARFSGSLLGGKAALTITGAQAEDEAEYYCVLWYSNLWVFGGGTKLTVLGQPKAAPSVTLFPPSSEELQANKATLVCLISDFYPGAVTVAWKADSSPVKAGVETTTPSKQSNNKYAASSYLSLTPEQWKSHRSYSCQVTHEGSTVEKTVAPTECS

SEQ ID NO: 59 - DNA, 645 bp, Homo sapiens
  source 1..645: mol_type = other DNA
caggctgtggtcacacaagagcctagcctgacagtgtctcctggcggcacagtgaccctgacctgtagatcttctacaggcgccgtgaccaccagcaactacgctaattgggtgcagcagaagcccggccaggctcctagaggactgatcggcggaacaaacaagagagccccttggacacccgccagattctctggatctctgctcggcggaaaggccgctctgacaatcactggtgctcaggctgaggacgaggccgagtactattgtgtgctgtggtacagcaacctgtgggtgttcggcggaggcaccaaactgacagttctgggtcagcccaaggcggcgccctcggtcactctgttcccgccctcctctgaggagcttcaagccaacaaggccacactggtgtgtctcataagtgacttctatccgggagccgtgacagtggcctggaaggcagatagcagccccgtcaaggcgggagtggagaccaccacaccctccaaacaaagcaacaacaagtacgcggccagcagctacctgagcctgacgcctgagcagtggaagtcccacagaagctacagctgccaggtcacgcatgaagggagcaccgtggagaagacagtggcccctacagaatgttca

SEQ ID NO: 60 - protein, 452 aa, Homo sapiens
EVQLVESGGGLVQPGGSLRLSCAASGFTFNTYAMNWVRQAPGKGLEWVGRIRSKYNNYATYYADSVKDRFTISRDDSKNSLYLQMNSLKTEDTAVYYCVRHGNFGNSYVSWFAYWGQGTLVTVSSASTKGPSVFPLAPCSRSTSESTAALGCLVKDYFPEPVTVSWNSGALTSGVHTFPAVLQSSGLYSLSSVVTVPSSSLGTKTYTCNVDHKPSNTKVDKRVESKYGPPCPPCPAPEFEGGPSVFLFPPKPKDTLMISRTPEVTCVVVDVSQEDPEVQFNWYVDGVEVHNAKTKPREEQFNSTYRVVSVLTVLHQDWLNGKEYKCKVSNKGLASSIEKTISKAKGQPREPQVYTLPPCQEEMTKNQVSLWCLVKGFYPSDIAVEWESNGQPENNYKTTPPVLDSDGSFFLYSKLTVDKSRWQEGNVFSCSVMHEALHNHYTQKSLSLSLGK

SEQ ID NO: 61 - DNA, 1356 bp, Homo sapiens
  source 1..1356: mol_type = other DNA
gaggtgcagctggttgaatctggcggaggactggttcagcctggcggatctctgagactgtcttgtgccgccagcggcttcaccttcaacacctacgctatgaactgggtccgacaggcccctggcaaaggactggaatgggtgggaagaatcaggtccaagtacaacaactacgccacctactacgccgacagcgtgaaggacagattcaccatcagcagggacgacagcaagaacagcctgtacctgcagatgaacagcctgaaaaccgaggacaccgccgtgtactactgtgtcagacacggcaacttcggcaacagctatgtgtcttggtttgcctactggggccagggcacactggtcacagttagctctgctagcaccaagggccccagcgtgttccccctggccccttgcagcagaagcaccagcgagagcacagccgccctgggctgcctggtgaaggactacttccccgagcccgtgaccgtgtcctggaacagcggcgctctgaccagcggcgtgcataccttccccgccgtgctccagagcagcggactgtactccctgagcagcgtggtgaccgtgccttccagcagcctgggcaccaagacctacacctgcaacgtggaccacaagcccagcaacaccaaggtggacaagagagtggagagcaagtacggccctccctgccccccttgccctgcccccgagttcgagggcggacctagcgtgttcctgttcccccccaagcccaaggacaccctgatgatcagcagaacccccgaggtgacctgcgtggtggtggacgtgtcccaggaggaccccgaggtccagtttaattggtacgtggacggcgtggaagtgcataacgccaagaccaagcccagagaggagcagttcaacagcacctacagagtggtgtccgtgctgaccgtgctgcaccaggactggctgaacggcaaggaatacaagtgcaaggtctccaacaagggcctggccagcagcatcgagaagaccatcagcaaggccaagggccagccacgggagccccaggtctacaccctgccaccttgtcaagaggagatgaccaagaaccaggtgtccctgtggtgtctggtgaaaggcttctatcccagcgatatcgccgtggagtgggagagcaacggccagcccgagaacaactacaagaccaccccccctgtgctggacagcgacggcagcttcttcctgtactccaagctgaccgtggacaagtccagatggcaggagggcaacgtcttcagctgctccgtgatgcacgaggccctgcacaaccactacacccagaagtccctgagcctgagcctgggcaag

SEQ ID NO: 62 - protein, 214 aa, Homo sapiens
EIVLTQSPGTLSLSPGERATLSCRASQSVSSYLAWYQKKPGQAPRLLIYDASNRATGIPDRFSGSGSGTDFTLTISRLEPEDFAVYYCQQRSNWPITFGQGTKLEIKRTVAAPSVFIFPPSDEQLKSGTASVVCLLNNFYPREAKVQWKVDNALQSGNSQESVTEQDSKDSTYSLSSTLTLSKADYEKHKVYACEVTHQGLSSPVTKSFNRGEC

SEQ ID NO: 63 - DNA, 642 bp, Homo sapiens
  source 1..642: mol_type = other DNA
gagatcgtgctgacacagagccctggcacactgtcactgtctccaggcgagagagccacactgagctgtagagccagccagagcgtgtcctcttacctggcctggtatcagaagaagcctggacaggctcccagactgctgatctacgacgccagcaacagagccacaggcatccccgatagattcagcggctctggctctggcaccgacttcaccctgacaatcagcagactggaacccgaggacttcgccgtgtactactgccagcagagaagcaactggcccatcacattcggccagggcaccaagctggaaatcaagcgaactgtggctgcaccatctgtcttcatcttcccgccatctgatgagcagttgaaatctggaactgcctctgttgtgtgcctgctgaataacttctatcccagagaggccaaagtacagtggaaggtggataacgccctccaatcgggtaactcccaggagagtgtcacagagcaggacagcaaggacagcacctacagcctcagcagcaccctgacgctgagcaaagcagactacgagaaacacaaagtctacgcctgcgaagtcacccatcagggcctgagctcgcccgtcacaaagagcttcaacaggggagagtgt

SEQ ID NO: 64 - protein, 449 aa, Homo sapiens
EVQLLESGGGVVQPGGSLRLSCAASGFTFNDYAMHWVREAPGKGLEWVSTISWNSGSIGYADSVKGRFTISRDNSKNTLYLQMNSLRAEDTAVYYCAKDIQYGNYYYGMDYWGQGTLVTVSSASTKGPSVFPLAPCSRSTSESTAALGCLVKDYFPEPVTVSWNSGALTSGVHTFPAVLQSSGLYSLSSVVTVPSSSLGTKTYTCNVDHKPSNTKVDKRVESKYGPPCPPCPAPEFEGGPSVFLFPPKPKDTLMISRTPEVTCVVVDVSQEDPEVQFNWYVDGVEVHNAKTKPREEQFNSTYRVVSVLTVLHQDWLNGKEYKCKVSNKGLASSIEKTISKAKGQPREPQVCTLPPSQEEMTKNQVSLSCAVKGFYPSDIAVEWESNGQPENNYKTTPPVLDSDGSFFLVSKLTVDKSRWQEGNVFSCSVMHEALHNHYTQKSLSLSLGK

SEQ ID NO: 65 - DNA, 1347 bp, Homo sapiens
  source 1..1347: mol_type = other DNA
gaagtgcagctgctggaatctggtggcggagttgttcagcctggcggctctctgagactgtcttgtgctgccagcggcttcaccttcaacgactacgctatgcactgggtccgagaggcccctggcaaaggacttgaatgggtgtccaccatcagctggaacagcggctctatcggctacgccgattccgtgaagggcagattcaccatctccagagacaacagcaagaacaccctgtacctgcagatgaacagcctgagagccgaggacaccgccgtgtactactgtgccaaggacatccagtacggcaactactactacggcatggactactggggccagggaacactggttaccgttagctctgctagcaccaagggccccagcgtgttccccctggccccttgcagcagaagcaccagcgagagcacagccgccctgggctgcctggtgaaggactacttccccgagcccgtgaccgtgtcctggaacagcggcgctctgaccagcggcgtgcataccttccccgccgtgctccagagcagcggactgtactccctgagcagcgtggtgaccgtgccttccagcagcctgggcaccaagacctacacctgcaacgtggaccacaagcccagcaacaccaaggtggacaagagagtggagagcaagtacggccctccctgccccccttgccctgcccccgagttcgagggcggacctagcgtgttcctgttcccccccaagcccaaggacaccctgatgatcagcagaacccccgaggtgacctgcgtggtggtggacgtgtcccaggaggaccccgaggtccagtttaattggtacgtggacggcgtggaagtgcataacgccaagaccaagcccagagaggagcagttcaacagcacctacagagtggtgtccgtgctgaccgtgctgcaccaggactggctgaacggcaaggaatacaagtgcaaggtctccaacaagggcctggccagcagcatcgagaagaccatcagcaaggccaagggccagccacgggagccccaggtctgcaccctgccacctagccaagaggagatgaccaagaaccaggtgtccctgagctgtgccgtgaaaggcttctatcccagcgatatcgccgtggagtgggagagcaacggccagcccgagaacaactacaagaccaccccccctgtgctggacagcgacggcagcttcttcctggtttccaagctgaccgtggacaagtccagatggcaggagggcaacgtcttcagctgctccgtgatgcacgaggccctgcacaaccactacacccagaagtccctgagcctgagcctgggcaag

SEQ ID NO: 66 - protein, 215 aa, Homo sapiens
QAVVTQEPSLTVSPGGTVTLTCRSSTGAVTTSNYANWVQEKPGQAPRGLIGGTNKRAPWTPARFSGSLLGGKAALTITGAQAEDEAEYYCVLWYSNLWVFGGGTKLTVLGQPKAAPSVTLFPPSSEELQANKATLVCLISDFYPGAVTVAWKADSSPVKAGVETTTPSKQSNNKYAASSYLSLTPEQWKSHRSYSCQVTHEGSTVEKTVAPTECS

SEQ ID NO: 67 - DNA, 645 bp, Homo sapiens
  source 1..645: mol_type = other DNA
caggctgtggtcacacaagagcctagcctgacagtgtctcctggcggcacagtgaccctgacctgtagatcttctacaggcgccgtgaccaccagcaactacgctaattgggtgcaggagaagcccggccaggctcctagaggactgatcggcggaacaaacaagagagccccttggacacccgccagattctctggatctctgctcggcggaaaggccgctctgacaatcactggtgctcaggctgaggacgaggccgagtactattgtgtgctgtggtacagcaacctgtgggtgttcggcggaggcaccaaactgacagttctgggtcagcccaaggcggcgccctcggtcactctgttcccgccctcctctgaggagcttcaagccaacaaggccacactggtgtgtctcataagtgacttctatccgggagccgtgacagtggcctggaaggcagatagcagccccgtcaaggcgggagtggagaccaccacaccctccaaacaaagcaacaacaagtacgcggccagcagctacctgagcctgacgcctgagcagtggaagtcccacagaagctacagctgccaggtcacgcatgaagggagcaccgtggagaagacagtggcccctacagaatgttca

SEQ ID NO: 68 - protein, 452 aa, Homo sapiens
EVQLVESGGGLVQPGGSLRLSCAASGFTFNTYAMNWVRKAPGKGLEWVGRIRSKYNNYATYYADSVKDRFTISRDDSKNSLYLQMNSLKTEDTAVYYCVRHGNFGNSYVSWFAYWGQGTLVTVSSASTKGPSVFPLAPCSRSTSESTAALGCLVKDYFPEPVTVSWNSGALTSGVHTFPAVLQSSGLYSLSSVVTVPSSSLGTKTYTCNVDHKPSNTKVDKRVESKYGPPCPPCPAPEFEGGPSVFLFPPKPKDTLMISRTPEVTCVVVDVSQEDPEVQFNWYVDGVEVHNAKTKPREEQFNSTYRVVSVLTVLHQDWLNGKEYKCKVSNKGLASSIEKTISKAKGQPREPQVYTLPPCQEEMTKNQVSLWCLVKGFYPSDIAVEWESNGQPENNYKTTPPVLDSDGSFFLYSKLTVDKSRWQEGNVFSCSVMHEALHNHYTQKSLSLSLGK

SEQ ID NO: 69 - DNA, 1356 bp, Homo sapiens
  source 1..1356: mol_type = other DNA
gaggtgcagctggttgaatctggcggaggactggttcagcctggcggatctctgagactgtcttgtgccgccagcggcttcaccttcaacacctacgctatgaactgggtccgaaaggcccctggcaaaggactggaatgggtgggaagaatcaggtccaagtacaacaactacgccacctactacgccgacagcgtgaaggacagattcaccatcagcagggacgacagcaagaacagcctgtacctgcagatgaacagcctgaaaaccgaggacaccgccgtgtactactgtgtcagacacggcaacttcggcaacagctatgtgtcttggtttgcctactggggccagggcacactggtcacagttagctctgctagcaccaagggccccagcgtgttccccctggccccttgcagcagaagcaccagcgagagcacagccgccctgggctgcctggtgaaggactacttccccgagcccgtgaccgtgtcctggaacagcggcgctctgaccagcggcgtgcataccttccccgccgtgctccagagcagcggactgtactccctgagcagcgtggtgaccgtgccttccagcagcctgggcaccaagacctacacctgcaacgtggaccacaagcccagcaacaccaaggtggacaagagagtggagagcaagtacggccctccctgccccccttgccctgcccccgagttcgagggcggacctagcgtgttcctgttcccccccaagcccaaggacaccctgatgatcagcagaacccccgaggtgacctgcgtggtggtggacgtgtcccaggaggaccccgaggtccagtttaattggtacgtggacggcgtggaagtgcataacgccaagaccaagcccagagaggagcagttcaacagcacctacagagtggtgtccgtgctgaccgtgctgcaccaggactggctgaacggcaaggaatacaagtgcaaggtctccaacaagggcctggccagcagcatcgagaagaccatcagcaaggccaagggccagccacgggagccccaggtctacaccctgccaccttgtcaagaggagatgaccaagaaccaggtgtccctgtggtgtctggtgaaaggcttctatcccagcgatatcgccgtggagtgggagagcaacggccagcccgagaacaactacaagaccaccccccctgtgctggacagcgacggcagcttcttcctgtactccaagctgaccgtggacaagtccagatggcaggagggcaacgtcttcagctgctccgtgatgcacgaggccctgcacaaccactacacccagaagtccctgagcctgagcctgggcaag

SEQ ID NO: 70 - protein, 214 aa, Homo sapiens
EIVLTQSPGTLSLSPGERATLSCRASQSVSSYLAWYQKKPGQAPRLLIYDASNRATGIPDRFSGSGSGTDFTLTISRLEPEDFAVYYCQQRSNWPITFGQGTKLEIKRTVAAPSVFIFPPSDKKLKSGTASVVCLLNNFYPREAKVQWKVDNALQSGNSQESVTEQDSKDSTYSLSSTLTLSKADYEKHKVYACEVTHQGLSSPVTKSFNRGEC

SEQ ID NO: 71 - DNA, 642 bp, Homo sapiens
  source 1..642: mol_type = other DNA
gagatcgtgctgacacagagccctggcacactgtcactgtctccaggcgagagagccacactgagctgtagagccagccagagcgtgtcctcttacctggcctggtatcagaagaagcctggacaggctcccagactgctgatctacgacgccagcaacagagccacaggcatccccgatagattcagcggctctggctctggcaccgacttcaccctgacaatcagcagactggaacccgaggacttcgccgtgtactactgccagcagagaagcaactggcccatcacattcggccagggcaccaagctggaaatcaagcgaactgtggctgcaccatctgtcttcatcttcccgccatctgataagaaattgaaatctggaactgcctctgttgtgtgcctgctgaataacttctatcccagagaggccaaagtacagtggaaggtggataacgccctccaatcgggtaactcccaggagagtgtcacagagcaggacagcaaggacagcacctacagcctcagcagcaccctgacgctgagcaaagcagactacgagaaacacaaagtctacgcctgcgaagtcacccatcagggcctgagctcgcccgtcacaaagagcttcaacaggggagagtgt

SEQ ID NO: 72 - protein, 449 aa, Homo sapiens
EVQLLESGGGVVQPGGSLRLSCAASGFTFNDYAMHWVREAPGKGLEWVSTISWNSGSIGYADSVKGRFTISRDNSKNTLYLQMNSLRAEDTAVYYCAKDIQYGNYYYGMDYWGQGTLVTVSSASTKGPSVFPLAPCSRSTSESTAALGCLVEDYFPEPVTVSWNSGALTSGVHTFPAVLQSSGLYSLSSVVTVPSSSLGTKTYTCNVDHKPSNTKVDERVESKYGPPCPPCPAPEFEGGPSVFLFPPKPKDTLMISRTPEVTCVVVDVSQEDPEVQFNWYVDGVEVHNAKTKPREEQFNSTYRVVSVLTVLHQDWLNGKEYKCKVSNKGLASSIEKTISKAKGQPREPQVCTLPPSQEEMTKNQVSLSCAVKGFYPSDIAVEWESNGQPENNYKTTPPVLDSDGSFFLVSKLTVDKSRWQEGNVFSCSVMHEALHNHYTQKSLSLSLGK

SEQ ID NO: 73 - DNA, 1347 bp, Homo sapiens
  source 1..1347: mol_type = other DNA
gaagtgcagctgctggaatctggtggcggagttgttcagcctggcggctctctgagactgtcttgtgctgccagcggcttcaccttcaacgactacgctatgcactgggtccgagaggcccctggcaaaggacttgaatgggtgtccaccatcagctggaacagcggctctatcggctacgccgattccgtgaagggcagattcaccatctccagagacaacagcaagaacaccctgtacctgcagatgaacagcctgagagccgaggacaccgccgtgtactactgtgccaaggacatccagtacggcaactactactacggcatggactactggggccagggaacactggttaccgttagctctgctagcaccaagggccccagcgtgttccccctggccccttgcagcagaagcaccagcgagagcacagccgccctgggctgcctggtggaggactacttccccgagcccgtgaccgtgtcctggaacagcggcgctctgaccagcggcgtgcataccttccccgccgtgctccagagcagcggactgtactccctgagcagcgtggtgaccgtgccttccagcagcctgggcaccaagacctacacctgcaacgtggaccacaagcccagcaacaccaaggtggacgagagagtggagagcaagtacggccctccctgccccccttgccctgcccccgagttcgaaggcggacctagcgtgttcctgttcccccccaagcccaaggacaccctgatgatcagcagaacccccgaggtgacctgcgtggtggtggacgtgtcccaggaggaccccgaggtccagtttaattggtacgtggacggcgtggaagtgcataacgccaagaccaagcccagagaggagcagttcaacagcacctacagagtggtgtccgtgctgaccgtgctgcaccaggactggctgaacggcaaggaatacaagtgcaaggtctccaacaagggcctggccagcagcatcgagaagaccatcagcaaggccaagggccagccacgggagccccaggtctgcaccctgccacctagccaagaggagatgaccaagaaccaggtgtccctgagctgtgccgtgaaaggcttctatcccagcgatatcgccgtggagtgggagagcaacggccagcccgagaacaactacaagaccaccccccctgtgctggacagcgacggcagcttcttcctggtttccaagctgaccgtggacaagtccagatggcaggagggcaacgtcttcagctgctccgtgatgcacgaggccctgcacaaccactacacccagaagtccctgagcctgagcctgggcaag

SEQ ID NO: 74 - protein, 449 aa, Homo sapiens
EVQLLESGGGVVQPGGSLRLSCAASGFTFNDYAMHWVREAPGKGLEWVSTISWNSGSIGYADSVKGRFTISRDNSKNTLYLQMNSLRAEDTAVYYCAKDIQYGNYYYGMDYWGQGTLVTVSSASTKGPSVFPLAPCSRSTSESTAALGCLVEDYFPEPVTVSWNSGALTSGVHTFPAVLQSSGLYSLSSVVTVPSSSLGTKTYTCNVDHKPSNTKVDERVESKYGPPCPPCPAPEFEGGPSVFLFPPKPKDTLMISRTPEVTCVVVDVSQEDPEVQFNWYVDGVEVHNAKTKPREEQFASTYRVVSVLTVLHQDWLNGKEYKCKVSNKGLPSSIEKTISKAKGQPREPQVCTLPPSQEEMTKNQVSLSCAVKGFYPSDIAVEWESNGQPENNYKTTPPVLDSDGSFFLVSKLTVDKSRWQEGNVFSCSVMHEALHNHYTQKSLSLSLGK

SEQ ID NO: 75 - DNA, 1347 bp, Homo sapiens
  source 1..1347: mol_type = other DNA
gaagtgcagctgctggaatctggtggcggagttgttcagcctggcggctctctgagactgtcttgtgctgccagcggcttcaccttcaacgactacgctatgcactgggtccgagaggcccctggcaaaggacttgaatgggtgtccaccatcagctggaacagcggctctatcggctacgccgattccgtgaagggcagattcaccatctccagagacaacagcaagaacaccctgtacctgcagatgaacagcctgagagccgaggacaccgccgtgtactactgtgccaaggacatccagtacggcaactactactacggcatggactactggggccagggaacactggttaccgttagctctgctagcaccaagggccccagcgtgttccccctggccccttgcagcagaagcaccagcgagagcacagccgccctgggctgcctggtggaggactacttccccgagcccgtgaccgtgtcctggaacagcggcgctctgaccagcggcgtgcataccttccccgccgtgctccagagcagcggactgtactccctgagcagcgtggtgaccgtgccttccagcagcctgggcaccaagacctacacctgcaacgtggaccacaagcccagcaacaccaaggtggacgagagagtggagagcaagtacggccctccctgccccccttgccctgcccccgagttcgaaggcggacctagcgtgttcctgttcccccccaagcccaaggacaccctgatgatcagcagaacccccgaggtgacctgcgtggtggtggacgtgtcccaggaggaccccgaggtccagtttaattggtacgtggacggcgtggaagtgcataacgccaagaccaagcccagagaggagcagttcgccagcacctacagagtggtgtccgtgctgaccgtgctgcaccaggactggctgaacggcaaggaatacaagtgcaaggtctccaacaagggcctgcctagcagcatcgagaagaccatcagcaaggccaagggccagccacgggagccccaggtctgcaccctgccacctagccaagaggagatgaccaagaaccaggtgtccctgagctgtgccgtgaaaggcttctatcccagcgatatcgccgtggagtgggagagcaacggccagcccgagaacaactacaagaccaccccccctgtgctggacagcgacggcagcttcttcctggtttccaagctgaccgtggacaagtccagatggcaggagggcaacgtcttcagctgctccgtgatgcacgaggccctgcacaaccactacacccagaagtccctgagcctgagcctgggcaag

SEQ ID NO: 76 - protein, 223 aa, Homo sapiens
EVQLVESGGGLVQPGGSLRLSCAASGFTFNTYAMNWVRKAPGKGLEWVGRIRSKYNNYATYYADSVKDRFTISRDDSKNSLYLQMNSLKTEDTAVYYCVRHGNFGNSYVSWFAYWGQGTLVTVSSASTKGPSVFPLAPCSRSTSESTAALGCLVKDYFPEPVTVSWNSGALTSGVHTFPAVLQSSGLYSLSSVVTVPSSSLGTKTYTCNVDHKPSNTKVDKRV

SEQ ID NO: 77 - DNA, 669 bp, Homo sapiens
  source 1..669: mol_type = other DNA
gaggtgcagctggttgaatctggcggaggactggttcagcctggcggatctctgagactgtcttgtgccgccagcggcttcaccttcaacacctacgctatgaactgggtccgaaaggcccctggcaaaggactggaatgggtgggaagaatcaggtccaagtacaacaactacgccacctactacgccgacagcgtgaaggacagattcaccatcagcagggacgacagcaagaacagcctgtacctgcagatgaacagcctgaaaaccgaggacaccgccgtgtactactgtgtcagacacggcaacttcggcaacagctatgtgtcttggtttgcctactggggccagggcacactggtcacagttagctctgctagcaccaagggccccagcgtgttccccctggccccttgcagcagaagcaccagcgagagcacagccgccctgggctgcctggtgaaggactacttccccgagcccgtgaccgtgtcctggaacagcggcgctctgaccagcggcgtgcataccttccccgccgtgctccagagcagcggactgtactccctgagcagcgtggtgaccgtgccttccagcagcctgggcaccaagacctacacctgcaacgtggaccacaagcccagcaacaccaaggtggacaagagagtg

SEQ ID NO: 78 - protein, 444 aa, Homo sapiens
QAVVTQEPSLTVSPGGTVTLTCRSSTGAVTTSNYANWVQEKPGQAPRGLIGGTNKRAPWTPARFSGSLLGGKAALTITGAQAEDEAEYYCVLWYSNLWVFGGGTKLTVLGQPKAAPSVTLFPPSSEELQANKATLVCLISDFYPGAVTVAWKADSSPVKAGVETTTPSKQSNNKYAASSYLSLTPEQWKSHRSYSCQVTHEGSTVEKTVAPTECSESKYGPPCPPCPAPEFEGGPSVFLFPPKPKDTLMISRTPEVTCVVVDVSQEDPEVQFNWYVDGVEVHNAKTKPREEQFASTYRVVSVLTVLHQDWLNGKEYKCKVSNKGLPSSIEKTISKAKGQPREPQVYTLPPCQEEMTKNQVSLWCLVKGFYPSDIAVEWESNGQPENNYKTTPPVLDSDGSFFLYSKLTVDKSRWQEGNVFSCSVMHEALHNHYTQKSLSLSLGK

SEQ ID NO: 79 - DNA, 1332 bp, Homo sapiens
  source 1..1332: mol_type = other DNA
caggctgtggtcacacaagagcctagcctgacagtgtctcctggcggcacagtgaccctgacctgtagatcttctacaggcgccgtgaccaccagcaactacgctaattgggtgcaggagaagcccggccaggctcctagaggactgatcggcggaacaaacaagagagccccttggacacccgccagattctctggatctctgctcggcggaaaggccgctctgacaatcactggtgctcaggctgaggacgaggccgagtactattgtgtgctgtggtacagcaacctgtgggtgttcggcggaggcaccaaactgacagttctgggtcagcccaaggcggcgccctcggtcactctgttcccgccctcctctgaggagcttcaagccaacaaggccacactggtgtgtctcataagtgacttctatccgggagccgtgacagtggcctggaaggcagatagcagccccgtcaaggcgggagtggagaccaccacaccctccaaacaaagcaacaacaagtacgcggccagcagctacctgagcctgacgcctgagcagtggaagtcccacagaagctacagctgccaggtcacgcatgaagggagcaccgtggagaagacagtggcccctacagaatgttcagagagcaagtacggccctccctgccccccttgccctgcccccgagttcgagggcggacctagcgtgttcctgttcccccccaagcccaaggacaccctgatgatcagcagaacccccgaggtgacctgcgtggtggtggacgtgtcccaggaggaccccgaggtccagtttaattggtacgtggacggcgtggaagtgcataacgccaagaccaagcccagagaggagcagttcgccagcacctacagagtggtgtccgtgctgaccgtgctgcaccaggactggctgaacggcaaggaatacaagtgcaaggtctccaacaagggcctgcctagcagcatcgagaagaccatcagcaaggccaagggccagccacgggagccccaggtctacaccctgccaccttgtcaagaggagatgaccaagaaccaggtgtccctgtggtgtctggtgaaaggcttctatcccagcgatatcgccgtggagtgggagagcaacggccagcccgagaacaactacaagaccaccccccctgtgctggacagcgacggcagcttcttcctgtactccaagctgaccgtggacaagtccagatggcaggagggcaacgtcttcagctgctccgtgatgcacgaggccctgcacaaccactacacccagaagtccctgagcctgagcctgggcaag

SEQ ID NO: 80 - protein, 218 aa, Homo sapiens
DIVLTQSPASLAVSPGQRATITCRASKSVSTSGYSYMHWYQKKPGQPPKLLIYLASNLESGVPARFSGSGSGTDFTLTINPVEAEDTANYYCQHSRELPWTFGQGTKVEIKRTVAAPSVFIFPPSDEQLKSGTASVVCLLNNFYPREAKVQWKVDNALQSGNSQESVTEQDSKDSTYSLSSTLTLSKADYEKHKVYACEVTHQGLSSPVTKSFNRGEC

SEQ ID NO: 81 - DNA, 654 bp, Homo sapiens
  source 1..654: mol_type = other DNA
gacatcgtgctgacacagagccctgcttctctggctgtgtctcctggccagagagccaccatcacctgtagagccagcaagagcgtgtccaccagcggctactcttacatgcactggtatcagaagaagcccggccagcctcctaagctgctgatctacctggctagcaacctcgaaagcggagtgcctgctagattttctggcagcggctctggcaccgacttcaccctgacaatcaaccccgtggaagccgaagacaccgccaactactactgccagcacagcagagagctgccctggacatttggccagggcaccaaggtggaaatcaagcgaactgtggctgcaccatctgtcttcatcttcccgccatctgatgagcagttgaaatctggaactgcctctgttgtgtgcctgctgaataacttctatcccagagaggccaaagtacagtggaaggtggataacgccctccaatcgggtaactcccaggagagtgtcacagagcaggacagcaaggacagcacctacagcctcagcagcaccctgacgctgagcaaagcagactacgagaaacacaaagtctacgcctgcgaagtcacccatcagggcctgagctcgcccgtcacaaagagcttcaacaggggagagtgt

SEQ ID NO: 82 - protein, 449 aa, Homo sapiens
QVQLVQSGSELKKPGASVKVSCKASGYIFTNFGMNWVREAPGQGLEWMGWINTYTGEQIYADGFTGRFVFSLDTSASTAYLQISSLKAEDTAVYFCARGEIYYGYDVGFVYWGQGTLVTVSSASTKGPSVFPLAPCSRSTSESTAALGCLVKDYFPEPVTVSWNSGALTSGVHTFPAVLQSSGLYSLSSVVTVPSSSLGTKTYTCNVDHKPSNTKVDKRVESKYGPPCPPCPAPEFEGGPSVFLFPPKPKDTLMISRTPEVTCVVVDVSQEDPEVQFNWYVDGVEVHNAKTKPREEQFNSTYRVVSVLTVLHQDWLNGKEYKCKVSNKGLASSIEKTISKAKGQPREPQVCTLPPSQEEMTKNQVSLSCAVKGFYPSDIAVEWESNGQPENNYKTTPPVLDSDGSFFLVSKLTVDKSRWQEGNVFSCSVMHEALHNHYTQKSLSLSLGK

SEQ ID NO: 83 - DNA, 1347 bp, Homo sapiens
  source 1..1347: mol_type = other DNA
caggttcagctggtgcagtctggcagcgagctgaagaaacctggcgcctctgtgaaggtgtcctgcaaggctagcggctacatcttcaccaacttcggcatgaactgggtccgagaggctcctggacagggactcgaatggatgggctggatcaacacctacaccggcgagcagatctacgccgatggcttcacaggcagattcgtgttcagcctggacaccagcgccagcacagcttacctgcagatcagctctctgaaggccgaggataccgccgtgtacttctgtgccagaggcgagatctactacggctacgacgtgggctttgtgtactggggccagggaacactggtcaccgttagctctgctagcaccaagggccccagcgtgttccccctggccccttgcagcagaagcaccagcgagagcacagccgccctgggctgcctggtgaaggactacttccccgagcccgtgaccgtgtcctggaacagcggcgctctgaccagcggcgtgcataccttccccgccgtgctccagagcagcggactgtactccctgagcagcgtggtgaccgtgccttccagcagcctgggcaccaagacctacacctgcaacgtggaccacaagcccagcaacaccaaggtggacaagagagtggagagcaagtacggccctccctgccccccttgccctgcccccgagttcgagggcggacctagcgtgttcctgttcccccccaagcccaaggacaccctgatgatcagcagaacccccgaggtgacctgcgtggtggtggacgtgtcccaggaggaccccgaggtccagtttaattggtacgtggacggcgtggaagtgcataacgccaagaccaagcccagagaggagcagttcaacagcacctacagagtggtgtccgtgctgaccgtgctgcaccaggactggctgaacggcaaggaatacaagtgcaaggtctccaacaagggcctggccagcagcatcgagaagaccatcagcaaggccaagggccagccacgggagccccaggtctgcaccctgccacctagccaagaggagatgaccaagaaccaggtgtccctgagctgtgccgtgaaaggcttctatcccagcgatatcgccgtggagtgggagagcaacggccagcccgagaacaactacaagaccaccccccctgtgctggacagcgacggcagcttcttcctggtttccaagctgaccgtggacaagtccagatggcaggagggcaacgtcttcagctgctccgtgatgcacgaggccctgcacaaccactacacccagaagtccctgagcctgagcctgggcaag

SEQ ID NO: 84 - protein, 218 aa, Homo sapiens
DIVLTQSPASLAVSPGQRATITCRASKSVTTSGYSYIHWYQKKPGQPPKLLIYLASDLEAGVPARFSGSGSGTDFTLTINPVEAEDTANYYCQHSRELPWTFGQGTKVEIKRTVAAPSVFIFPPSDEQLKSGTASVVCLLNNFYPREAKVQWKVDNALQSGNSQESVTEQDSKDSTYSLSSTLTLSKADYEKHKVYACEVTHQGLSSPVTKSFNRGEC

SEQ ID NO: 85 - DNA, 654 bp, Homo sapiens
  source 1..654: mol_type = other DNA
gacatcgtgctgacacagagccctgcttctctggctgtgtctcctggccagagagccaccatcacctgtagagccagcaagagcgtgaccaccagcggctactcttacatccactggtatcagaagaagcccggccagcctcctaagctgctgatctacctggccagcgatctggaagctggcgtgccagctagattttctggcagcggctctggcaccgacttcaccctgacaatcaaccccgtggaagccgaagacaccgccaactactactgccagcacagcagagagctgccctggacatttggccagggcaccaaggtggaaatcaagcgaactgtggctgcaccatctgtcttcatcttcccgccatctgatgagcagttgaaatctggaactgcctctgttgtgtgcctgctgaataacttctatcccagagaggccaaagtacagtggaaggtggataacgccctccaatcgggtaactcccaggagagtgtcacagagcaggacagcaaggacagcacctacagcctcagcagcaccctgacgctgagcaaagcagactacgagaaacacaaagtctacgcctgcgaagtcacccatcagggcctgagctcgcccgtcacaaagagcttcaacaggggagagtgt

SEQ ID NO: 86 - protein, 449 aa, Homo sapiens
QVQLVQSGSELKKPGASVKVSCKASGYIFTNFGMNWVREAPGQGLEWMGWINTYTGEQIYADGFTGRFVFSLDTSVSTAYLQISSLKAEDTAVYFCARGEIYYGYDVGFVYWGQGTLVTVSSASTKGPSVFPLAPCSRSTSESTAALGCLVKDYFPEPVTVSWNSGALTSGVHTFPAVLQSSGLYSLSSVVTVPSSSLGTKTYTCNVDHKPSNTKVDKRVESKYGPPCPPCPAPEFEGGPSVFLFPPKPKDTLMISRTPEVTCVVVDVSQEDPEVQFNWYVDGVEVHNAKTKPREEQFNSTYRVVSVLTVLHQDWLNGKEYKCKVSNKGLASSIEKTISKAKGQPREPQVCTLPPSQEEMTKNQVSLSCAVKGFYPSDIAVEWESNGQPENNYKTTPPVLDSDGSFFLVSKLTVDKSRWQEGNVFSCSVMHEALHNHYTQKSLSLSLGK

SEQ ID NO: 87 - DNA, 1347 bp, Homo sapiens
  source 1..1347: mol_type = other DNA
caggttcagctggtgcagtctggcagcgagctgaagaaacctggcgcctctgtgaaggtgtcctgcaaggctagcggctacatcttcaccaacttcggcatgaactgggtccgagaggctcctggacagggactcgaatggatgggctggatcaacacctacaccggcgagcagatctacgccgatggcttcacaggcagattcgtgttcagcctggacaccagcgtcagcacagcttacctgcagatcagctctctgaaggccgaggataccgccgtgtacttctgtgccagaggcgagatctactacggctacgacgtgggctttgtgtactggggccagggaacactggtcaccgttagctctgctagcaccaagggccccagcgtgttccccctggccccttgcagcagaagcaccagcgagagcacagccgccctgggctgcctggtgaaggactacttccccgagcccgtgaccgtgtcctggaacagcggcgctctgaccagcggcgtgcataccttccccgccgtgctccagagcagcggactgtactccctgagcagcgtggtgaccgtgccttccagcagcctgggcaccaagacctacacctgcaacgtggaccacaagcccagcaacaccaaggtggacaagagagtggagagcaagtacggccctccctgccccccttgccctgcccccgagttcgagggcggacctagcgtgttcctgttcccccccaagcccaaggacaccctgatgatcagcagaacccccgaggtgacctgcgtggtggtggacgtgtcccaggaggaccccgaggtccagtttaattggtacgtggacggcgtggaagtgcataacgccaagaccaagcccagagaggagcagttcaacagcacctacagagtggtgtccgtgctgaccgtgctgcaccaggactggctgaacggcaaggaatacaagtgcaaggtctccaacaagggcctggccagcagcatcgagaagaccatcagcaaggccaagggccagccacgggagccccaggtctgcaccctgccacctagccaagaggagatgaccaagaaccaggtgtccctgagctgtgccgtgaaaggcttctatcccagcgatatcgccgtggagtgggagagcaacggccagcccgagaacaactacaagaccaccccccctgtgctggacagcgacggcagcttcttcctggtttccaagctgaccgtggacaagtccagatggcaggagggcaacgtcttcagctgctccgtgatgcacgaggccctgcacaaccactacacccagaagtccctgagcctgagcctgggcaag

SEQ ID NO: 88 - protein, 219 aa, Homo sapiens
DVVMTQSPLSLPVTPGEPASISCRSSQSIVHSNGNTYLEWYLKKPGQSPQLLIYKVSNRFSGVPDRFSGSGSGTDFTLKISRVEAEDVGVYFCLQVTHVPLTFGQGTKLEIKRTVAAPSVFIFPPSDEQLKSGTASVVCLLNNFYPREAKVQWKVDNALQSGNSQESVTEQDSKDSTYSLSSTLTLSKADYEKHKVYACEVTHQGLSSPVTKSFNRGEC

SEQ ID NO: 89 - DNA, 657 bp, Homo sapiens
  source 1..657: mol_type = other DNA
gacgtggtcatgacacagagccctctgagcctgcctgtgacacctggcgaacctgccagcatcagctgtagaagcagccagagcatcgtgcacagcaacggcaacacatacctggagtggtatctgaagaagcccggccagtctcctcagctgctgatctacaaggtgtccaacagattcagcggcgtgcccgacagattctctggctctggatctggcaccgacttcaccctgaagatctccagagtggaagccgaggacgtgggcgtgtacttctgtctccaggtcacacacgtgcccctgacatttggccagggcaccaagctggaaatcaagcgaactgtggctgcaccatctgtcttcatcttcccgccatctgatgagcagttgaaatctggaactgcctctgttgtgtgcctgctgaataacttctatcccagagaggccaaagtacagtggaaggtggataacgccctccaatcgggtaactcccaggagagtgtcacagagcaggacagcaaggacagcacctacagcctcagcagcaccctgacgctgagcaaagcagactacgagaaacacaaagtctacgcctgcgaagtcacccatcagggcctgagctcgcccgtcacaaagagcttcaacaggggagagtgt

SEQ ID NO: 90 - protein, 442 aa, Homo sapiens
QVQLVQSGAEVKKPGSSVKVSCKASGYTFADYEIHWVREAPGQGLEWMGAIHPGSGGTAYAQKFQGRVTLTADESSTTAYMELSSLRSEDTAVYYCTRYYSFAYWGQGTLVTVSSASTKGPSVFPLAPCSRSTSESTAALGCLVKDYFPEPVTVSWNSGALTSGVHTFPAVLQSSGLYSLSSVVTVPSSSLGTKTYTCNVDHKPSNTKVDKRVESKYGPPCPPCPAPEFEGGPSVFLFPPKPKDTLMISRTPEVTCVVVDVSQEDPEVQFNWYVDGVEVHNAKTKPREEQFNSTYRVVSVLTVLHQDWLNGKEYKCKVSNKGLASSIEKTISKAKGQPREPQVCTLPPSQEEMTKNQVSLSCAVKGFYPSDIAVEWESNGQPENNYKTTPPVLDSDGSFFLVSKLTVDKSRWQEGNVFSCSVMHEALHNHYTQKSLSLSLGK

SEQ ID NO: 91 - DNA, 1326 bp, Homo sapiens
  source 1..1326: mol_type = other DNA
caggttcagctggttcagtctggcgccgaagtgaagaaacctggcagcagcgtgaaggtgtcctgcaaggctagcggctacaccttcgccgactacgagatccactgggtccgagaggctccaggacagggacttgaatggatgggcgctatccatcctggctctggcggcacagcttacgcccagaaattccagggcagagtgaccctgaccgccgacgagtctagcaccaccgcctacatggaactgagcagcctgagaagcgaggacaccgccgtgtactactgcacccggtactacagcttcgcctactggggacagggaaccctggtcacagtcagctctgctagcaccaagggccccagcgtgttccccctggccccttgcagcagaagcaccagcgagagcacagccgccctgggctgcctggtgaaggactacttccccgagcccgtgaccgtgtcctggaacagcggcgctctgaccagcggcgtgcataccttccccgccgtgctccagagcagcggactgtactccctgagcagcgtggtgaccgtgccttccagcagcctgggcaccaagacctacacctgcaacgtggaccacaagcccagcaacaccaaggtggacaagagagtggagagcaagtacggccctccctgccccccttgccctgcccccgagttcgagggcggacctagcgtgttcctgttcccccccaagcccaaggacaccctgatgatcagcagaacccccgaggtgacctgcgtggtggtggacgtgtcccaggaggaccccgaggtccagtttaattggtacgtggacggcgtggaagtgcataacgccaagaccaagcccagagaggagcagttcaacagcacctacagagtggtgtccgtgctgaccgtgctgcaccaggactggctgaacggcaaggaatacaagtgcaaggtctccaacaagggcctggccagcagcatcgagaagaccatcagcaaggccaagggccagccacgggagccccaggtctgcaccctgccacctagccaagaggagatgaccaagaaccaggtgtccctgagctgtgccgtgaaaggcttctatcccagcgatatcgccgtggagtgggagagcaacggccagcccgagaacaactacaagaccaccccccctgtgctggacagcgacggcagcttcttcctggtttccaagctgaccgtggacaagtccagatggcaggagggcaacgtcttcagctgctccgtgatgcacgaggccctgcacaaccactacacccagaagtccctgagcctgagcctgggcaag

SEQ ID NO: 92 - protein, 219 aa, Homo sapiens
DVVMTQSPLSLPVTPGEPASISCRSSQSIVHSNGNTYLEWYLKKPGQSPQLLIYKVSNRFSGVPDRFSGSGSGTDFTLKISRVEAEDVGVYFCLQVTHVPLTFGQGTKLEIKRTVAAPSVFIFPPSDKKLKSGTASVVCLLNNFYPREAKVQWKVDNALQSGNSQESVTEQDSKDSTYSLSSTLTLSKADYEKHKVYACEVTHQGLSSPVTKSFNRGEC

SEQ ID NO: 93 - DNA, 657 bp, Homo sapiens
  source 1..657: mol_type = other DNA
gacgtggtcatgacacagagccctctgagcctgcctgtgacacctggcgaacctgccagcatcagctgtagaagcagccagagcatcgtgcacagcaacggcaacacatacctggagtggtatctgaagaagcccggccagtctcctcagctgctgatctacaaggtgtccaacagattcagcggcgtgcccgacagattctctggctctggatctggcaccgacttcaccctgaagatctccagagtggaagccgaggacgtgggcgtgtacttctgtctccaggtcacacacgtgcccctgacatttggccagggcaccaagctggaaatcaagcgaactgtggctgcaccatctgtcttcatcttcccgccatctgataagaaattgaaatctggaactgcctctgttgtgtgcctgctgaataacttctatcccagagaggccaaagtacagtggaaggtggataacgccctccaatcgggtaactcccaggagagtgtcacagagcaggacagcaaggacagcacctacagcctcagcagcaccctgacgctgagcaaagcagactacgagaaacacaaagtctacgcctgcgaagtcacccatcagggcctgagctcgcccgtcacaaagagcttcaacaggggagagtgt

SEQ ID NO: 94 - protein, 442 aa, Homo sapiens
QVQLVQSGAEVKKPGSSVKVSCKASGYTFADYEIHWVREAPGQGLEWMGAIHPGSGGTAYAQKFQGRVTLTADESSTTAYMELSSLRSEDTAVYYCTRYYSFAYWGQGTLVTVSSASTKGPSVFPLAPCSRSTSESTAALGCLVEDYFPEPVTVSWNSGALTSGVHTFPAVLQSSGLYSLSSVVTVPSSSLGTKTYTCNVDHKPSNTKVDERVESKYGPPCPPCPAPEFEGGPSVFLFPPKPKDTLMISRTPEVTCVVVDVSQEDPEVQFNWYVDGVEVHNAKTKPREEQFNSTYRVVSVLTVLHQDWLNGKEYKCKVSNKGLASSIEKTISKAKGQPREPQVCTLPPSQEEMTKNQVSLSCAVKGFYPSDIAVEWESNGQPENNYKTTPPVLDSDGSFFLVSKLTVDKSRWQEGNVFSCSVMHEALHNHYTQKSLSLSLGK

SEQ ID NO: 95 - DNA, 1326 bp, Homo sapiens
  source 1..1326: mol_type = other DNA
caggttcagctggttcagtctggcgccgaagtgaagaaacctggcagcagcgtgaaggtgtcctgcaaggctagcggctacaccttcgccgactacgagatccactgggtccgagaggctccaggacagggacttgaatggatgggcgctatccatcctggctctggcggcacagcttacgcccagaaattccagggcagagtgaccctgaccgccgacgagtctagcaccaccgcctacatggaactgagcagcctgagaagcgaggacaccgccgtgtactactgcacccggtactacagcttcgcctactggggacagggaaccctggtcacagtcagctctgctagcaccaagggccccagcgtgttccccctggccccttgcagcagaagcaccagcgagagcacagccgccctgggctgcctggtggaggactacttccccgagcccgtgaccgtgtcctggaacagcggcgctctgaccagcggcgtgcataccttccccgccgtgctccagagcagcggactgtactccctgagcagcgtggtgaccgtgccttccagcagcctgggcaccaagacctacacctgcaacgtggaccacaagcccagcaacaccaaggtggacgagagagtggagagcaagtacggccctccctgccccccttgccctgcccccgagttcgaaggcggacctagcgtgttcctgttcccccccaagcccaaggacaccctgatgatcagcagaacccccgaggtgacctgcgtggtggtggacgtgtcccaggaggaccccgaggtccagtttaattggtacgtggacggcgtggaagtgcataacgccaagaccaagcccagagaggagcagttcaacagcacctacagagtggtgtccgtgctgaccgtgctgcaccaggactggctgaacggcaaggaatacaagtgcaaggtctccaacaagggcctggccagcagcatcgagaagaccatcagcaaggccaagggccagccacgggagccccaggtctgcaccctgccacctagccaagaggagatgaccaagaaccaggtgtccctgagctgtgccgtgaaaggcttctatcccagcgatatcgccgtggagtgggagagcaacggccagcccgagaacaactacaagaccaccccccctgtgctggacagcgacggcagcttcttcctggtttccaagctgaccgtggacaagtccagatggcaggagggcaacgtcttcagctgctccgtgatgcacgaggccctgcacaaccactacacccagaagtccctgagcctgagcctgggcaag

SEQ ID NO: 96 - protein, 6 aa, synthetic construct
ADYEIH

SEQ ID NO: 97 - protein, 17 aa, synthetic construct
AIHPGSGGTAYAQKFQG

SEQ ID NO: 98 - protein, 6 aa, synthetic construct
YYSFAY

SEQ ID NO: 99 - protein, 115 aa, synthetic construct
QVQLVQSGAEVKKPGSSVKVSCKASGYTFADYEIHWVRQAPGQGLEWMGAIHPGSGGTAYAQKFQGRVTLTADESSTTAYMELSSLRSEDTAVYYCTRYYSFAYWGQGTLVTVSS

SEQ ID NO: 100 - DNA, 345 bp, synthetic construct
  source 1..345: mol_type = other DNA
caggttcagctggttcagtctggcgccgaagtgaagaaacctggcagcagcgtgaaggtgtcctgcaaggctagcggctacaccttcgccgactacgagatccactgggtccgagaggctccaggacagggacttgaatggatgggcgctatccatcctggctctggcggcacagcttacgcccagaaattccagggcagagtgaccctgaccgccgacgagtctagcaccaccgcctacatggaactgagcagcctgagaagcgaggacaccgccgtgtactactgcacccggtactacagcttcgcctactggggacagggaaccctggtcacagtcagctct

SEQ ID NO: 101 - protein, 16 aa, synthetic construct
RSSQSIVHSNGNTYLE

SEQ ID NO: 102 - protein, 7 aa, synthetic construct
KVSNRFS

SEQ ID NO: 103 - protein, 9 aa, synthetic construct
LQVTHVPLT

SEQ ID NO: 104 - protein, 112 aa, synthetic construct
DVVMTQSPLSLPVTPGEPASISCRSSQSIVHSNGNTYLEWYLQKPGQSPQLLIYKVSNRFSGVPDRFSGSGSGTDFTLKISRVEAEDVGVYFCLQVTHVPLTFGQGTKLEIK

SEQ ID NO: 105 - DNA, 336 bp, synthetic construct
  source 1..336: mol_type = other DNA
gacgtggtcatgacacagagccctctgagcctgcctgtgacacctggcgaacctgccagcatcagctgtagaagcagccagagcatcgtgcacagcaacggcaacacatacctggagtggtatctgaagaagcccggccagtctcctcagctgctgatctacaaggtgtccaacagattcagcggcgtgcccgacagattctctggctctggatctggcaccgacttcaccctgaagatctccagagtggaagccgaggacgtgggcgtgtacttctgtctccaggtcacacacgtgcccctgacatttggccagggcaccaagctggaaatcaag